European Patent Application EP 4 733 388 A1, published April 29, 2026. Title: 鼠李糖乳杆菌菌株、活菌制剂及其制备方法和用途. Applicant: 科郦有限公司. The sequence listing filed with the application follows.

SEQUENCE LISTING (9 sequences)

SEQ ID NO: 1 - DNA, 1439 bp, Lactobacillus rhamnosus
  source 1..1439: mol_type = other DNA
  misc_feature 1..1403: note = 16S rRNA gene
tgcagtcgaacgagttctgattattgaaaggtgcttgcatcttgatttaattttgaacgagtggcggacgggtgagtaacacgtgggtaacctgcccttaagtgggggataacatttggaaacagatgctaataccgcataaatccaagaaccgcatggttcttggctgaaagatggcgtaagctatcgcttttggatggacccgcggcgtattagctagttggtgaggtaacggctcaccaaggcaatgatacgtagccgaactgagaggttgatcggccacattgggactgagacacggcccaaactcctacgggaggcagcagtagggaatcttccacaatggacgcaagtctgatggagcaacgccgcgtgagtgaagaaggctttcgggtcgtaaaactctgttgttggagaagaatggtcggcagagtaactgttgtcggcgtgacggtatccaaccagaaagccacggctaactacgtgccagcagccgcggtaatacgtaggtggcaagcgttatccggatttattgggcgtaaagcgagcgcaggcggttttttaagtctgatgtgaaagccctcggcttaaccgaggaagtgcatcggaaactgggaaacttgagtgcagaagaggacagtggaactccatgtgtagcggtgaaatgcgtagatatatggaagaacaccagtggcgaaggcggctgtctggtctgtaactgacgctgaggctcgaaagcatgggtagcgaacaggattagataccctggtagtccatgccgtaaacgatgaatgctaggtgttggagggtttccgcccttcagtgccgcagctaacgcattaagcattccgcctggggagtacgaccgcaaggttgaaactcaaaggaattgacgggggcccgcacaagcggtggagcatgtggtttaattcgaagcaacgcgaagaaccttaccaggtcttgacatcttttgatcacctgagagatcaggtttccccttcgggggcaaaatgacaggtggtgcatggttgtcgtcagctcgtgtcgtgagatgttgggttaagtcccgcaacgagcgcaacccttatgactagttgccagcatttagttgggcactctagtaagactgccggtgacaaaccggaggaaggtggggatgacgtcaaatcatcatgccccttatgacctgggctacacacgtgctacaatggatggtacaacgagttgcgagaccgcgaggtcaagctaatctcttaaagccattctcagttcggactgtaggctgcaactcgcctacacgaagtcggaatcgctagtaatcgcggatcagcacgccgcggtgaatacgttcccgggccttgtacacaccgcccgtcacaccatgagagtttgtaacacccgaagccggtggcgtaacccttttagggagcgagccgtct

SEQ ID NO: 2 - DNA, 10 bp, synthetic construct
  source 1..10: mol_type = other DNA
  misc_feature 1..10: note = OPA-02 primer
tgccgagctg

SEQ ID NO: 3 - DNA, 10 bp, synthetic construct
  source 1..10: mol_type = other DNA
  misc_feature 1..10: note = OPA-18 primer
aggtgaccgt

SEQ ID NO: 4 - DNA, 10 bp, synthetic construct
  source 1..10: mol_type = other DNA
  misc_feature 1..10: note = OPL-07 primer
aggcgggaac

SEQ ID NO: 5 - DNA, 10 bp, synthetic construct
  source 1..10: mol_type = other DNA
  misc_feature 1..10: note = OPL-16 primer
aggttgcagg

SEQ ID NO: 6 - DNA, 10 bp, synthetic construct
  source 1..10: mol_type = other DNA
  misc_structure 1..10: note = OPM-05 primer
gggaacgtgt

SEQ ID NO: 7 - DNA, 18 bp, synthetic construct
  source 1..18: mol_type = other DNA
  misc_feature 1..18: note = 27F primer
agtttgatcmtggctcag

SEQ ID NO: 8 - DNA, 19 bp, synthetic construct
  source 1..19: mol_type = other DNA
  misc_feature 1..19: note = 1492R primer
ggttaccttgttacgactt

SEQ ID NO: 9 - DNA, 395 bp, Lactobacillus rhamnosus
  source 1..395: mol_type = other DNA
  misc_feature 1..395: note = pheS gene
cgccatatacatcggcgtcaatattagccgcacgtaaaacattcggatgcaccatgccggcaccgagaacttcaatccagccggtatacttgcaaacagggcagcccttgccaccgcagcggaagcaggaaacgtccacttctacagacggttctgtaaacggaaaatagctcgggcgcaggcgaatcgtccgatcagcgccaaacacatgctgacacatggcgagtaacgtccccttaagatcagccattgtaatatgcttgtcgatcaccaggccttccattgatggaactggtggctatgtgtggcatcatcatcatcacgccgataaaccacgcctggactgatcattttcagcgggcccttagtaaagtcatgtttctccatcgtccgcg